European Patent Specification EP 3 688 023 B1, published August 27, 2025. Title: METHODS AND COMPOSITIONS FOR CANCER TREATMENT. Applicant: Dingfu Biotarget Co., Ltd. The sequence listing filed with the application follows.

SEQUENCE LISTING (91 sequences)

SEQ ID NO: 1 - protein, 227 aa, Artificial Sequence
  Y349C+T366W
DKTHTCPPCPAPELLGGPSVFLFPPKPKDTLMISRTPEVTCVVVDVSHENPEVKFNWYVDGVEVHNAKTKPREEQYNSTYRVVSVLTVLHQDWLNGKEYKCKVSNKALPAPIEKTISKAKGQPREPQVCTLPPSRDELTKNQVSLWCLVKGFYPSDIAVEWESNGQPENNYKTTPPVLDSDGSFFLYSKLTVDKSRWQQGNVFSCSVMHEALHNHYTQKSLSLSPGK

SEQ ID NO: 2 - protein, 227 aa, Artificial Sequence
  D356C+T366S+L368A+Y407V+F405K
DKTHTCPPCPAPELLGGPSVFLFPPKPKDTLMISRTPEVTCVVVDVSHEDPEVKFNWYVDGVEVHNAKTKPREEQYNSTYRVVSVLTVLHQDWLNGKEYKCKVSNKALPAPIEKTISKAKGQPREPQVYTLPPSRCELTKNQVSLSCAVKGFYPSDIAVEWESNGQPENNYKTTPPVLDSDGSFKLVSKLTVDKSRWQQGNVFSCSVMHEALHNHYTQKSLSLSPGK

SEQ ID NO: 3 - protein, 227 aa, Artificial Sequence
  Y349C+T366W+F405K
DKTHTCPPCPAPELLGGPSVFLFPPKPKDTLMISRTPEVTCVVVDVSHENPEVKFNWYVDGVEVHNAKTKPREEQYNSTYRVVSVLTVLHQDWLNGKEYKCKVSNKALPAPIEKTISKAKGQPREPQVCTLPPSRDELTKNQVSLWCLVKGFYPSDIAVEWESNGQPENNYKTTPPVLDSDGSFKLYSKLTVDKSRWQQGNVFSCSVMHEALHNHYTQKSLSLSPGK

SEQ ID NO: 4 - protein, 227 aa, Artificial Sequence
  D356C+T366S+L368A+Y407V
DKTHTCPPCPAPELLGGPSVFLFPPKPKDTLMISRTPEVTCVVVDVSHEDPEVKFNWYVDGVEVHNAKTKPREEQYNSTYRVVSVLTVLHQDWLNGKEYKCKVSNKALPAPIEKTISKAKGQPREPQVYTLPPSRCELTKNQVSLSCAVKGFYPSDIAVEWESNGQPENNYKTTPPVLDSDGSFFLVSKLTVDKSRWQQGNVFSCSVMHEALHNHYTQKSLSLSPGK

SEQ ID NO: 5 - protein, 227 aa, Artificial Sequence
  Y349C+T366W+K409E
DKTHTCPPCPAPELLGGPSVFLFPPKPKDTLMISRTPEVTCVVVDVSHENPEVKFNWYVDGVEVHNAKTKPREEQYNSTYRVVSVLTVLHQDWLNGKEYKCKVSNKALPAPIEKTISKAKGQPREPQVCTLPPSRDELTKNQVSLWCLVKGFYPSDIAVEWESNGQPENNYKTTPPVLDSDGSFFLYSELTVDKSRWQQGNVFSCSVMHEALHNHYTQKSLSLSPGK

SEQ ID NO: 6 - protein, 227 aa, Artificial Sequence
  Y349C+T366W+K409A
DKTHTCPPCPAPELLGGPSVFLFPPKPKDTLMISRTPEVTCVVVDVSHENPEVKFNWYVDGVEVHNAKTKPREEQYNSTYRVVSVLTVLHQDWLNGKEYKCKVSNKALPAPIEKTISKAKGQPREPQVCTLPPSRDELTKNQVSLWCLVKGFYPSDIAVEWESNGQPENNYKTTPPVLDSDGSFFLYSALTVDKSRWQQGNVFSCSVMHEALHNHYTQKSLSLSPGK

SEQ ID NO: 7 - protein, 227 aa, Artificial Sequence
  Y349C+T366W+F405K+K360E+Q347E
DKTHTCPPCPAPELLGGPSVFLFPPKPKDTLMISRTPEVTCVVVDVSHENPEVKFNWYVDGVEVHNAKTKPREEQYNSTYRVVSVLTVLHQDWLNGKEYKCKVSNKALPAPIEKTISKAKGQPREPEVCTLPPSRDELTENQVSLWCLVKGFYPSDIAVEWESNGQPENNYKTTPPVLDSDGSFKLYSKLTVDKSRWQQGNVFSCSVMHEALHNHYTQKSLSLSPGK

SEQ ID NO: 8 - protein, 227 aa, Artificial Sequence
  D356C+T366S+L368A+Y407V+Q347R
DKTHTCPPCPAPELLGGPSVFLFPPKPKDTLMISRTPEVTCVVVDVSHEDPEVKFNWYVDGVEVHNAKTKPREEQYNSTYRVVSVLTVLHQDWLNGKEYKCKVSNKALPAPIEKTISKAKGQPREPRVYTLPPSRCELTKNQVSLSCAVKGFYPSDIAVEWESNGQPENNYKTTPPVLDSDGSFFLVSKLTVDKSRWQQGNVFSCSVMHEALHNHYTQKSLSLSPGK

SEQ ID NO: 9 - protein, 227 aa, Artificial Sequence
  Y349C+T366W+F405K+Q347R
DKTHTCPPCPAPELLGGPSVFLFPPKPKDTLMISRTPEVTCVVVDVSHENPEVKFNWYVDGVEVHNAKTKPREEQYNSTYRVVSVLTVLHQDWLNGKEYKCKVSNKALPAPIEKTISKAKGQPREPRVCTLPPSRDELTKNQVSLWCLVKGFYPSDIAVEWESNGQPENNYKTTPPVLDSDGSFKLYSKLTVDKSRWQQGNVFSCSVMHEALHNHYTQKSLSLSPGK

SEQ ID NO: 10 - protein, 227 aa, Artificial Sequence
  D356C+T366S+L368A+Y407V+K360E+Q347E
DKTHTCPPCPAPELLGGPSVFLFPPKPKDTLMISRTPEVTCVVVDVSHEDPEVKFNWYVDGVEVHNAKTKPREEQYNSTYRVVSVLTVLHQDWLNGKEYKCKVSNKALPAPIEKTISKAKGQPREPEVYTLPPSRCELTENQVSLSCAVKGFYPSDIAVEWESNGQPENNYKTTPPVLDSDGSFFLVSKLTVDKSRWQQGNVFSCSVMHEALHNHYTQKSLSLSPGK

SEQ ID NO: 11 - protein, 227 aa, Artificial Sequence
  Y349C+T366W+K409A+K360E+Q347E
DKTHTCPPCPAPELLGGPSVFLFPPKPKDTLMISRTPEVTCVVVDVSHENPEVKFNWYVDGVEVHNAKTKPREEQYNSTYRVVSVLTVLHQDWLNGKEYKCKVSNKALPAPIEKTISKAKGQPREPEVCTLPPSRDELTENQVSLWCLVKGFYPSDIAVEWESNGQPENNYKTTPPVLDSDGSFFLYSALTVDKSRWQQGNVFSCSVMHEALHNHYTQKSLSLSPGK

SEQ ID NO: 12 - protein, 227 aa, Artificial Sequence
  D356C+T366S+L368A+Y407V+F405K+Q347R
DKTHTCPPCPAPELLGGPSVFLFPPKPKDTLMISRTPEVTCVVVDVSHEDPEVKFNWYVDGVEVHNAKTKPREEQYNSTYRVVSVLTVLHQDWLNGKEYKCKVSNKALPAPIEKTISKAKGQPREPRVYTLPPSRCELTKNQVSLSCAVKGFYPSDIAVEWESNGQPENNYKTTPPVLDSDGSFKLVSKLTVDKSRWQQGNVFSCSVMHEALHNHYTQKSLSLSPGK

SEQ ID NO: 13 - protein, 227 aa, Artificial Sequence
  Y349C+T366W+K409A+Q347R
DKTHTCPPCPAPELLGGPSVFLFPPKPKDTLMISRTPEVTCVVVDVSHENPEVKFNWYVDGVEVHNAKTKPREEQYNSTYRVVSVLTVLHQDWLNGKEYKCKVSNKALPAPIEKTISKAKGQPREPRVCTLPPSRDELTKNQVSLWCLVKGFYPSDIAVEWESNGQPENNYKTTPPVLDSDGSFFLYSALTVDKSRWQQGNVFSCSVMHEALHNHYTQKSLSLSPGK

SEQ ID NO: 14 - protein, 227 aa, Artificial Sequence
  D356C+T366S+L368A+Y407V+F405K+K360E+Q347E
DKTHTCPPCPAPELLGGPSVFLFPPKPKDTLMISRTPEVTCVVVDVSHEDPEVKFNWYVDGVEVHNAKTKPREEQYNSTYRVVSVLTVLHQDWLNGKEYKCKVSNKALPAPIEKTISKAKGQPREPEVYTLPPSRCELTENQVSLSCAVKGFYPSDIAVEWESNGQPENNYKTTPPVLDSDGSFKLVSKLTVDKSRWQQGNVFSCSVMHEALHNHYTQKSLSLSPGK

SEQ ID NO: 15 - protein, 227 aa, Artificial Sequence
  T366W+K409A+K392D
DKTHTCPPCPAPELLGGPSVFLFPPKPKDTLMISRTPEVTCVVVDVSHENPEVKFNWYVDGVEVHNAKTKPREEQYNSTYRVVSVLTVLHQDWLNGKEYKCKVSNKALPAPIEKTISKAKGQPREPQVYTLPPSRDELTKNQVSLWCLVKGFYPSDIAVEWESNGQPENNYDTTPPVLDSDGSFFLYSALTVDKSRWQQGNVFSCSVMHEALHNHYTQKSLSLSPGK

SEQ ID NO: 16 - protein, 227 aa, Artificial Sequence
  T366S+L368A+Y407V+D399S+F405K
DKTHTCPPCPAPELLGGPSVFLFPPKPKDTLMISRTPEVTCVVVDVSHEDPEVKFNWYVDGVEVHNAKTKPREEQYNSTYRVVSVLTVLHQDWLNGKEYKCKVSNKALPAPIEKTISKAKGQPREPQVYTLPPSRDELTKNQVSLSCAVKGFYPSDIAVEWESNGQPENNYKTTPPVLSSDGSFKLVSKLTVDKSRWQQGNVFSCSVMHEALHNHYTQKSLSLSPGK

SEQ ID NO: 17 - protein, 227 aa, Artificial Sequence
  T366W+K409A
DKTHTCPPCPAPELLGGPSVFLFPPKPKDTLMISRTPEVTCVVVDVSHENPEVKFNWYVDGVEVHNAKTKPREEQYNSTYRVVSVLTVLHQDWLNGKEYKCKVSNKALPAPIEKTISKAKGQPREPQVYTLPPSRDELTKNQVSLWCLVKGFYPSDIAVEWESNGQPENNYKTTPPVLDSDGSFFLYSALTVDKSRWQQGNVFSCSVMHEALHNHYTQKSLSLSPGK

SEQ ID NO: 18 - protein, 227 aa, Artificial Sequence
  T366S+L368G+Y407A+F405K
DKTHTCPPCPAPELLGGPSVFLFPPKPKDTLMISRTPEVTCVVVDVSHEDPEVKFNWYVDGVEVHNAKTKPREEQYNSTYRVVSVLTVLHQDWLNGKEYKCKVSNKALPAPIEKTISKAKGQPREPQVYTLPPSRDELTKNQVSLSCGVKGFYPSDIAVEWESNGQPENNYKTTPPVLDSDGSFKLASKLTVDKSRWQQGNVFSCSVMHEALHNHYTQKSLSLSPGK

SEQ ID NO: 19 - protein, 227 aa, Artificial Sequence
  T366W+K409A+Y349D
DKTHTCPPCPAPELLGGPSVFLFPPKPKDTLMISRTPEVTCVVVDVSHENPEVKFNWYVDGVEVHNAKTKPREEQYNSTYRVVSVLTVLHQDWLNGKEYKCKVSNKALPAPIEKTISKAKGQPREPQVDTLPPSRDELTKNQVSLWCLVKGFYPSDIAVEWESNGQPENNYKTTPPVLDSDGSFFLYSALTVDKSRWQQGNVFSCSVMHEALHNHYTQKSLSLSPGK

SEQ ID NO: 20 - protein, 227 aa, Artificial Sequence
  T366S+L368A+Y407V+F405K+E357A
DKTHTCPPCPAPELLGGPSVFLFPPKPKDTLMISRTPEVTCVVVDVSHEDPEVKFNWYVDGVEVHNAKTKPREEQYNSTYRVVSVLTVLHQDWLNGKEYKCKVSNKALPAPIEKTISKAKGQPREPQVYTLPPSRDALTKNQVSLSCAVKGFYPSDIAVEWESNGQPENNYKTTPPVLDSDGSFKLVSKLTVDKSRWQQGNVFSCSVMHEALHNHYTQKSLSLSPGK

SEQ ID NO: 21 - protein, 227 aa, Artificial Sequence
  T366W+K409A+Y349D+S354D
DKTHTCPPCPAPELLGGPSVFLFPPKPKDTLMISRTPEVTCVVVDVSHENPEVKFNWYVDGVEVHNAKTKPREEQYNSTYRVVSVLTVLHQDWLNGKEYKCKVSNKALPAPIEKTISKAKGQPREPQVDTLPPDRDELTKNQVSLWCLVKGFYPSDIAVEWESNGQPENNYKTTPPVLDSDGSFFLYSALTVDKSRWQQGNVFSCSVMHEALHNHYTQKSLSLSPGK

SEQ ID NO: 22 - protein, 227 aa, Artificial Sequence
  T366W+F405K
DKTHTCPPCPAPELLGGPSVFLFPPKPKDTLMISRTPEVTCVVVDVSHENPEVKFNWYVDGVEVHNAKTKPREEQYNSTYRVVSVLTVLHQDWLNGKEYKCKVSNKALPAPIEKTISKAKGQPREPQVYTLPPSRDELTKNQVSLWCLVKGFYPSDIAVEWESNGQPENNYKTTPPVLDSDGSFKLYSKLTVDKSRWQQGNVFSCSVMHEALHNHYTQKSLSLSPGK

SEQ ID NO: 23 - protein, 227 aa, Artificial Sequence
  T366S+L368A+Y407V+K409A
DKTHTCPPCPAPELLGGPSVFLFPPKPKDTLMISRTPEVTCVVVDVSHEDPEVKFNWYVDGVEVHNAKTKPREEQYNSTYRVVSVLTVLHQDWLNGKEYKCKVSNKALPAPIEKTISKAKGQPREPQVYTLPPSRDELTKNQVSLSCAVKGFYPSDIAVEWESNGQPENNYKTTPPVLDSDGSFFLVSALTVDKSRWQQGNVFSCSVMHEALHNHYTQKSLSLSPGK

SEQ ID NO: 24 - protein, 227 aa, Artificial Sequence
  T366W+F405K+D399S
DKTHTCPPCPAPELLGGPSVFLFPPKPKDTLMISRTPEVTCVVVDVSHENPEVKFNWYVDGVEVHNAKTKPREEQYNSTYRVVSVLTVLHQDWLNGKEYKCKVSNKALPAPIEKTISKAKGQPREPQVYTLPPSRDELTKNQVSLWCLVKGFYPSDIAVEWESNGQPENNYKTTPPVLSSDGSFKLYSKLTVDKSRWQQGNVFSCSVMHEALHNHYTQKSLSLSPGK

SEQ ID NO: 25 - protein, 227 aa, Artificial Sequence
  T366S+L368A+Y407V+K409A+K392D
DKTHTCPPCPAPELLGGPSVFLFPPKPKDTLMISRTPEVTCVVVDVSHEDPEVKFNWYVDGVEVHNAKTKPREEQYNSTYRVVSVLTVLHQDWLNGKEYKCKVSNKALPAPIEKTISKAKGQPREPQVYTLPPSRDELTKNQVSLSCAVKGFYPSDIAVEWESNGQPENNYDTTPPVLDSDGSFFLVSALTVDKSRWQQGNVFSCSVMHEALHNHYTQKSLSLSPGK

SEQ ID NO: 26 - protein, 227 aa, Artificial Sequence
  T366W+F405K
DKTHTCPPCPAPELLGGPSVFLFPPKPKDTLMISRTPEVTCVVVDVSHEDPEVKFNWYVDGVEVHNAKTKPREEQYNSTYRVVSVLTVLHQDWLNGKEYKCKVSNKALPAPIEKTISKAKGQPREPQVYTLPPSRDELTKNQVSLSCGVKGFYPSDIAVEWESNGQPENNYKTTPPVLDSDGSFFLASALTVDKSRWQQGNVFSCSVMHEALHNHYTQKSLSLSPGK

SEQ ID NO: 27 - protein, 227 aa, Artificial Sequence
  T366S+L368G+Y407A+K409A
DKTHTCPPCPAPELLGGPSVFLFPPKPKDTLMISRTPEVTCVVVDVSHENPEVKFNWYVDGVEVHNAKTKPREEQYNSTYRVVSVLTVLHQDWLNGKEYKCKVSNKALPAPIEKTISKAKGQPREPQVDTLPPSRDELTKNQVSLWCLVKGFYPSDIAVEWESNGQPENNYKTTPPVLDSDGSFKLYSKLTVDKSRWQQGNVFSCSVMHEALHNHYTQKSLSLSPGK

SEQ ID NO: 28 - protein, 227 aa, Artificial Sequence
  T366W +F405K +Y349D
DKTHTCPPCPAPELLGGPSVFLFPPKPKDTLMISRTPEVTCVVVDVSHEDPEVKFNWYVDGVEVHNAKTKPREEQYNSTYRVVSVLTVLHQDWLNGKEYKCKVSNKALPAPIEKTISKAKGQPREPQVYTLPPSRDALTKNQVSLSCAVKGFYPSDIAVEWESNGQPENNYKTTPPVLDSDGSFFLVSALTVDKSRWQQGNVFSCSVMHEALHNHYTQKSLSLSPGK

SEQ ID NO: 29 - protein, 227 aa, Artificial Sequence
  T366S+L368A+Y407V +K409A +E357A
DKTHTCPPCPAPELLGGPSVFLFPPKPKDTLMISRTPEVTCVVVDVSHENPEVKFNWYVDGVEVHNAKTKPREEQYNSTYRVVSVLTVLHQDWLNGKEYKCKVSNKALPAPIEKTISKAKGQPREPQVDTLPPDRDELTKNQVSLWCLVKGFYPSDIAVEWESNGQPENNYKTTPPVLDSDGSFKLYSKLTVDKSRWQQGNVFSCSVMHEALHNHYTQKSLSLSPGK

SEQ ID NO: 30 - protein, 227 aa, Artificial Sequence
  wildtype human IgG1-Fc region amino acid
DKTHTCPPCPAPELLGGPSVFLFPPKPKDTLMISRTPEVTCVVVDVSHEDPEVKFNWYVDGVEVHNAKTKPREEQYNSTYRVVSVLTVLHQDWLNGKEYKCKVSNKALPAPIEKTISKAKGQPREPQVYTLPPSRDELTKNQVSLTCLVKGFYPSDIAVEWESNGQPENNYKTTPPVLDSDGSFFLYSKLTVDKSRWQQGNVFSCSVMHEALHNHYTQKSLSLSPGK

SEQ ID NO: 31 - DNA, 681 bp, Artificial Sequence
  Fc gene fragment
gacaagacccacacctgccccccctgccccgcccccgagctgctgggcggccccagcgtgttcctgttcccccccaagcccaaggacaccctgatgatcagccgcacccccgaggtgacctgcgtggtggtggacgtgagccacgagaaccccgaggtgaagttcaactggtacgtggacggcgtggaggtgcacaacgccaagaccaagccccgcgaggagcagtacaacagcacctaccgcgtggtgagcgtgctgaccgtgctgcaccaggactggctgaacggcaaggagtacaagtgcaaggtgagcaacaaggccctgcccgcccccatcgagaagaccatcagcaaggccaagggccagccccgcgagccccaggtgtacaccctgccccccagccgcgacgagctgaccaagaaccaggtgagcctgacctgcctggtgaagggcttctaccccagcgacatcgccgtggagtgggagagcaacggccagcccgagaacaactacaagaccaccccccccgtgctggacagcgacggcagcttcttcctgtacagcaagctgaccgtggacaagagccgctggcagcagggcaacgtgttcagctgcagcgtgatgcacgaggccctgcacaaccactacacccagaagagcctgagcctgagccccggcaag

SEQ ID NO: 32 - DNA, 741 bp, Artificial Sequence
  polynucleotide fragment encoding a mouse kappaIII signal peptide
atggagaccgacaccctgctgctgtgggtgctgctgctgtgggtgcccggcagcaccggcgacaagacccacacctgccccccctgccccgcccccgagctgctgggcggccccagcgtgttcctgttcccccccaagcccaaggacaccctgatgatcagccgcacccccgaggtgacctgcgtggtggtggacgtgagccacgagaaccccgaggtgaagttcaactggtacgtggacggcgtggaggtgcacaacgccaagaccaagccccgcgaggagcagtacaacagcacctaccgcgtggtgagcgtgctgaccgtgctgcaccaggactggctgaacggcaaggagtacaagtgcaaggtgagcaacaaggccctgcccgcccccatcgagaagaccatcagcaaggccaagggccagccccgcgagccccaggtgtacaccctgccccccagccgcgacgagctgaccaagaaccaggtgagcctgacctgcctggtgaagggcttctaccccagcgacatcgccgtggagtgggagagcaacggccagcccgagaacaactacaagaccaccccccccgtgctggacagcgacggcagcttcttcctgtacagcaagctgaccgtggacaagagccgctggcagcagggcaacgtgttcagctgcagcgtgatgcacgaggccctgcacaaccactacacccagaagagcctgagcctgagccccggcaag

SEQ ID NO: 33 - DNA, 1473 bp, Artificial Sequence
  gene  of ScFv-Fc fusion protein
atggagaccgacaccctgctgctgtgggtgctgctgctgtgggtgcccggcagcaccggcgaggtgcagctgctggagagcggcggcggcgtggtgcagcccggccgcagcctgcgcctgagctgcatcgccagcggcttcaccttcagcagctaccccatgacctgggtgcgccaggcccccggcaagggcctggagtgggtggccagcatcagctacgacggcagctacaagtacaaggccgacagcatgaagggccgcctgaccatcagccgcgacaacagcaagaacaccctgtacctggagatgaacagcctgaccgccgaggacaccgccgtgtactactgcgcccgcaccgccttcttcaacgcctacgacttctggggccagggcaccctggtgaccgtgagcagcgccagcaccaagggccccagcgtgggcggcggcggcagcggcggcggcggcagcgagatcgtgatgacccagagccccgccaccctgagcgtgagccccggcgagcgcgccaccctgagctgccgcgccagccagagcgtgcgcagcaacctggcctggtaccagcagaagcccggccaggccccccgcctgctgatctacgccgccagcacccgcgccaccggcatccccgcccgcttcagcggcagcggcagcggcaccgagttcaccctgaccatcagcagcctgcagagcgaggacttcgccgtgtactactgccagcagtacaacgagtggttccgcaccagcggccagggcaccaaggtggagatcaagcgcgacaagacccacacctgccccccctgccccgcccccgagctgctgggcggccccagcgtgttcctgttcccccccaagcccaaggacaccctgatgatcagccgcacccccgaggtgacctgcgtggtggtggacgtgagccacgagaaccccgaggtgaagttcaactggtacgtggacggcgtggaggtgcacaacgccaagaccaagccccgcgaggagcagtacaacagcacctaccgcgtggtgagcgtgctgaccgtgctgcaccaggactggctgaacggcaaggagtacaagtgcaaggtgagcaacaaggccctgcccgcccccatcgagaagaccatcagcaaggccaagggccagccccgcgagccccaggtgtacaccctgccccccagccgcgacgagctgaccaagaaccaggtgagcctgacctgcctggtgaagggcttctaccccagcgacatcgccgtggagtgggagagcaacggccagcccgagaacaactacaagaccaccccccccgtgctggacagcgacggcagcttcttcctgtacagcaagctgaccgtggacaagagccgctggcagcagggcaacgtgttcagctgcagcgtgatgcacgaggccctgcacaaccactacacccagaagagcctgagcctgagccccggcaag

SEQ ID NO: 34 - protein, 471 aa, Artificial Sequence
  ScFv-Fc fusion protein
EVQLLESGGGVVQPGRSLRLSCIASGFTFSSYPMTWVRQAPGKGLEWVASISYDGSYKYKADSMKGRLTISRDNSKNTLYLEMNSLTAEDTAVYYCARTAFFNAYDFWGQGTLVTVSSASTKGPSVGGGGSGGGGSEIVMTQSPATLSVSPGERATLSCRASQSVRSNLAWYQQKPGQAPRLLIYAASTRATGIPARFSGSGSGTEFTLTISSLQSEDFAVYYCQQYNEWFRTSGQGTKVEIKRDKTHTCPPCPAPELLGGPSVFLFPPKPKDTLMISRTPEVTCVVVDVSHENPEVKFNWYVDGVEVHNAKTKPREEQYNSTYRVVSVLTVLHQDWLNGKEYKCKVSNKALPAPIEKTISKAKGQPREPQVYTLPPSRDELTKNQVSLTCLVKGFYPSDIAVEWESNGQPENNYKTTPPVLDSDGSFFLYSKLTVDKSRWQQGNVFSCSVMHEALHNHYTQKSLSLSPGK

SEQ ID NO: 35 - DNA, 1121 bp, Artificial Sequence
  a fusion gene fragment encoding the fusion protein VhH-Fc
atggagaccgacaccctgctgctgtgggtgctgctgctgtgggtgcccggcagcaccggccaggtgcagctgcaggagtctgggggaggctcggtgcaggctggagggtctctgagactctcctgtgcagcctctgaatacatctacagtagctactgcatggcctggttccgccaggctccagggaaggagcgcgagggggtcgcagttattgggagtgatggtagcacaagctacgcagactccgtgaaaggccgattcaccatctccaaagacaacgccaagaacactctgtatctgcaaatgaacagcctgaaacctgaggacactgccatgtactactgtgcggccatcggtggttactgctaccaaccaccctatgagtaccagtactggggccaggggacccaggtcaccgtctcccagaaccgaaaagcagcgacaagacccacacctgccccccctgccccgcccccgagctgctgggcggccccagcgtgttcctgttcccccccaagcccaaggacaccctgatgatcagccgcacccccgaggtgacctgcgtggtggtggacgtgagccacgagaaccccgaggtgaagttcaactggtacgtggacggcgtggaggtgcacaacgccaagaccaagccccgcgaggagcagtacaacagcacctaccgcgtggtgagcgtgctgaccgtgctgcaccaggactggctgaacggcaaggagtacaagtgcaaggtgagcaacaaggccctgcccgcccccatcgagaagaccatcagcaaggccaagggccagccccgcgagccccaggtgtacaccctgccccccagccgcgacgagctgaccaagaaccaggtgagcctgacctgcctggtgaagggcttctaccccagcgacatcgccgtggagtgggagagcaacggccagcccgagaacaactacaagaccaccccccccgtgctggacagcgacggcagcttcttcctgtacagcaagctgaccgtggacaagagccgctggcagcagggcaacgtgttcagctgcagcgtgatgcacgaggccctgcacaaccactacacccagaagagcctgagcctgagccccggcaag

SEQ ID NO: 36 - protein, 354 aa, Artificial Sequence
  fusion protein VhH-Fc
QVQLQESGGGSVQAGGSLRLSCAASEYIYSSYCMAWFRQAPGKEREGVAVIGSDGSTSYADSVKGRFTISKDNAKNTLYLQMNSLKPEDTAMYYCAAIGGYCYQPPYEYQYWGQGTQVTVSSEPKSSDKTHTCPPCPAPELLGGPSVFLFPPKPKDTLMISRTPEVTCVVVDVSHEDPEVKFNWYVDGVEVHNAKTKPREEQYNSTYRVVSVLTVLHQDWLNGKEYKCKVSNKALPAPIEKTISKAKGQPREPQVYTLPPSRDELTKNQVSLTCLVKGFYPSDIAVEWESNGQPENNYKTTPPVLDSDGSFFLYSKLTVDKSRWQQGNVFSCSVMHEALHNHYTQKSLSLSPGK

SEQ ID NO: 37 - protein, 214 aa, Artificial Sequence
  amino acid sequence of Erb-LC
DILLTQSPVILSVSPGERVSFSCRASQSIGTNIHWYQQRTNGSPRLLIKYASESISGIPSRFSGSGSGTDFTLSINSVESEDIADYYCQQNNNWPTTFGAGTKLELKRTVAAPSVFIFPPSDEQLKSGTASVVCLLNNFYPREAKVQWKVDNALQSGNSQESVTEQDSKDSTYSLSSTLTLSKADYEKHKVYACEVTHQGLSSPVTKSFNRGEC

SEQ ID NO: 38 - DNA, 642 bp, Artificial Sequence
  gene of Erb-LC
gacatcctgctgacccagagccccgtgatcctgagcgtgagccccggcgagcgcgtgagcttcagctgccgcgccagccagagcatcggcaccaacatccactggtaccagcagcgcaccaacggcagcccccgcctgctgatcaagtacgccagcgagagcatcagcggcatccccagccgcttcagcggcagcggcagcggcaccgacttcaccctgagcatcaacagcgtggagagcgaggacatcgccgactactactgccagcagaacaacaactggcccaccaccttcggcgccggcaccaagctggagctgaagcgcaccgtggccgcccccagcgtgttcatcttcccccccagcgacgagcagctgaagagcggcaccgccagcgtggtgtgcctgctgaacaacttctacccccgcgaggccaaggtgcagtggaaggtggacaacgccctgcagagcggcaacagccaggagagcgtgaccgagcaggacagcaaggacagcacctacagcctgagcagcaccctgaccctgagcaaggccgactacgagaagcacaaggtgtacgcctgcgaggtgacccaccagggcctgagcagccccgtgaccaagagcttcaaccgcggcgagtgc

SEQ ID NO: 39 - protein, 449 aa, Artificial Sequence
  amino acid sequences of Erb-Fc9
QVQLKQSGPGLVQPSQSLSITCTVSGFSLTNYGVHWVRQSPGKGLEWLGVIWSGGNTDYNTPFTSRLSINKDNSKSQVFFKMNSLQSNDTAIYYCARALTYYDYEFAYWGQGTLVTVSAASTKGPSVFPLAPSSKSTSGGTAALGCLVKDYFPEPVTVSWNSGALTSGVHTFPAVLQSSGLYSLSSVVTVPSSSLGTQTYICNVNHKPSNTKVDKRVEPKSCDKTHTCPPCPAPELLGGPSVFLFPPKPKDTLMISRTPEVTCVVVDVSHEDPEVKFNWYVDGVEVHNAKTKPREEQYNSTYRVVSVLTVLHQDWLNGKEYKCKVSNKALPAPIEKTISKAKGQPREPQVYTLPPSRDELTKNQVSLWCLVKGFYPSDIAVEWESNGQPENNYKTTPPVLDSDGSFFLYSALTVDKSRWQQGNVFSCSVMHEALHNHYTQKSLSLSPGK

SEQ ID NO: 40 - DNA, 1347 bp, Artificial Sequence
  gene of Erb-Fc9
caggtgcagctgaagcagagcggccccggcctggtgcagcccagccagagcctgagcatcacctgcaccgtgagcggcttcagcctgaccaactacggcgtgcactgggtgcgccagagccccggcaagggcctggagtggctgggcgtgatctggagcggcggcaacaccgactacaacacccccttcaccagccgcctgagcatcaacaaggacaacagcaagagccaggtgttcttcaagatgaacagcctgcagagcaacgacaccgccatctactactgcgcccgcgccctgacctactacgactacgagttcgcctactggggccagggcaccctggtgaccgtgagcgccgccagcactaaggggccctctgtgtttccactcgccccttctagcaaaagcacttccggaggaactgccgctctgggctgtctggtgaaagattacttccccgaaccagtcactgtgtcatggaactctggagcactgacatctggagttcacacctttcctgctgtgctgcagagttctggactgtactccctgtcatctgtggtcaccgtgccatcttcatctctggggacccagacctacatctgtaacgtgaaccacaaaccctccaacacaaaagtggacaaacgagtcgaaccaaaatcttgtgacaaaacccacacatgcccaccgtgcccagctccggaactcctgggcggaccgtcagtcttcctcttccccccaaaacccaaggacaccctcatgatctcccggacccctgaggtcacatgcgtggtggtggacgtgagccacgaagaccctgaggtcaagttcaactggtacgtggacggcgtggaggtgcataatgccaagacaaagccgcgggaggagcagtacaacagcacgtaccgtgtggtcagcgtcctcaccgtcctgcaccaggactggctgaatggcaaggagtacaagtgcaaggtctccaacaaagccctcccagcccccatcgagaaaaccatctccaaagccaaagggcagccccgagaaccacaggtgtacaccctgcccccaagtcgggatgagctgaccaagaaccaggtcagcctgtggtgcctggtcaaaggcttctatcccagcgacatcgccgtggagtgggagagcaatgggcagccggagaacaactacaagaccacgcctcccgtgttggactccgacggctccttcttcctctacagcgcgctcaccgtggacaagagcaggtggcagcaggggaacgtcttctcatgctccgtgatgcatgaggctctgcacaaccactacacgcagaagagcctctccctgtctccgggtaaa

SEQ ID NO: 41 - protein, 214 aa, Artificial Sequence
  amino acid sequence of T-LC
DIQMTQSPSSLSASVGDRVTITCRASQDVNTAVAWYQQKPGKAPKLLIYSASFLYSGVPSRFSGSRSGTDFTLTISSLQPEDFATYYCQQHYTTPPTFGQGTKVEIKRTVAAPSVFIFPPSDEQLKSGTASVVCLLNNFYPREAKVQWKVDNALQSGNSQESVTEQDSKDSTYSLSSTLTLSKADYEKHKVYACEVTHQGLSSPVTKSFNRGEC

SEQ ID NO: 42 - DNA, 708 bp, Artificial Sequence
  gene of T-LC
gacatccagatgacccagagccccagcagcctgagcgccagcgtgggcgaccgcgtgaccatcacctgccgcgccagccaggacgtgaacaccgccgtggcctggtaccagcagaagcccggcaaggcccccaagctgctgatctacagcgccagcttcctgtacagcggcgtgcccagccgcttcagcggcagccgcagcggcaccgacttcaccctgaccatcagcagcctgcagcccgaggacttcgccacctactactgccagcagcactacaccaccccccccaccttcggccagggcaccaaggtggagatcaaatactactgccagcagaacaacaactggcccaccaccttcggcgccggcaccaagctggagctgaagcgcaccgtggccgcccccagcgtgttcatcttcccccccagcgacgagcagctgaagagcggcaccgccagcgtggtgtgcctgctgaacaacttctacccccgcgaggccaaggtgcagtggaaggtggacaacgccctgcagagcggcaacagccaggagagcgtgaccgagcaggacagcaaggacagcacctacagcctgagcagcaccctgaccctgagcaaggccgactacgagaagcacaaggtgtacgcctgcgaggtgacccaccagggcctgagcagccccgtgaccaagagcttcaaccgcggcgagtgc

SEQ ID NO: 43 - protein, 450 aa, Artificial Sequence
  amino acid sequences of T-Fc9
EVQLVESGGGLVQPGGSLRLSCAASGFNIKDTYIHWVRQAPGKGLEWVARIYPTNGYTRYADSVKGRFTISADTSKNTAYLQMNSLRAEDTAVYYCSRWGGDGFYAMDYWGQGTLVTVSSASTKGPSVFPLAPSSKSTSGGTAALGCLVKDYFPEPVTVSWNSGALTSGVHTFPAVLQSSGLYSLSSVVTVPSSSLGTQTYICNVNHKPSNTKVDKRVEPKSCDKTHTCPPCPAPELLGGPSVFLFPPKPKDTLMISRTPEVTCVVVDVSHEDPEVKFNWYVDGVEVHNAKTKPREEQYNSTYRVVSVLTVLHQDWLNGKEYKCKVSNKALPAPIEKTISKAKGQPREPQVYTLPPSRDELTKNQVSLWCLVKGFYPSDIAVEWESNGQPENNYKTTPPVLDSDGSFFLYSALTVDKSRWQQGNVFSCSVMHEALHNHYTQKSLSLSPGK

SEQ ID NO: 44 - DNA, 1350 bp, Artificial Sequence
  gene of T-Fc9
gaggtgcagctggtggagagcggcggcggcctggtgcagcccggcggcagcctgcgcctgagctgcgccgccagcggcttcaacatcaaggacacctacatccactgggtgcgccaggcccccggcaagggcctggagtgggtggcccgcatctaccccaccaacggctacacccgctacgccgacagcgtgaagggccgcttcaccatcagcgccgacaccagcaagaacaccgcctacctgcagatgaacagcctgcgcgccgaggacaccgccgtgtactactgcagccgctggggcggcgacggcttctacgccatggactactggggccagggcaccctggtgaccgtgagcagcgccagcactaaggggccctctgtgtttccactcgccccttctagcaaaagcacttccggaggaactgccgctctgggctgtctggtgaaagattacttccccgaaccagtcactgtgtcatggaactctggagcactgacatctggagttcacacctttcctgctgtgctgcagagttctggactgtactccctgtcatctgtggtcaccgtgccatcttcatctctggggacccagacctacatctgtaacgtgaaccacaaaccctccaacacaaaagtggacaaacgagtcgaaccaaaatcttgtgacaaaacccacacatgcccaccgtgcccagctccggaactcctgggcggaccgtcagtcttcctcttccccccaaaacccaaggacaccctcatgatctcccggacccctgaggtcacatgcgtggtggtggacgtgagccacgaagaccctgaggtcaagttcaactggtacgtggacggcgtggaggtgcataatgccaagacaaagccgcgggaggagcagtacaacagcacgtaccgtgtggtcagcgtcctcaccgtcctgcaccaggactggctgaatggcaaggagtacaagtgcaaggtctccaacaaagccctcccagcccccatcgagaaaaccatctccaaagccaaagggcagccccgagaaccacaggtgtacaccctgcccccaagtcgggatgagctgaccaagaaccaggtcagcctgtggtgcctggtcaaaggcttctatcccagcgacatcgccgtggagtgggagagcaatgggcagccggagaacaactacaagaccacgcctcccgtgttggactccgacggctccttcttcctctacagcgcgctcaccgtggacaagagcaggtggcagcaggggaacgtcttctcatgctccgtgatgcatgaggctctgcacaaccactacacgcagaagagcctctccctgtctccgggtaaa

SEQ ID NO: 45 - protein, 215 aa, Artificial Sequence
  amino acid sequence of 28H1-LC
EIVLTQSPGTLSLSPGERATLSCRASQSVSRSYLAWYQQKPGQAPRLLIIGASTRATGIPDRFSGSGSGTDFTLTISRLEPEDFAVYYCQQGQVIPPTFGQGTKVEIKRTVAAPSVFIFPPSDEQLKSGTASVVCLLNNFYPREAKVQWKVDNALQSGNSQESVTEQDSKDSTYSLSSTLTLSKADYEKHKVYACEVTHQGLSSPVTKSFNRGEC

SEQ ID NO: 46 - DNA, 645 bp, Artificial Sequence
  gene of 28H1-LC
gagatcgtgctgacacagtctccaggcaccctgtctctgtctccaggagagagagccaccctgtcttgcagagcctctcagagcgtgtccaggagctacctggcttggtatcagcagaagccaggacaggcccctagactgctgatcatcggagcctctacaagagccacaggcatcccagacagattcagcggcagcggaagcggcacagacttcaccctgaccatcagcaggctggagccagaggacttcgccgtgtactattgccagcagggccaggtcatccctcctacctttggacagggcaccaaggtggagatcaagcgtacggtggctgcaccatctgtcttcatcttcccgccatctgatgagcagttgaaatctggtaccgctagcgttgtgtgcctgctgaataacttttatccacgggaggctaaggtgcagtggaaagtggacaatgccctccagagcggaaatagccaagagtccgttaccgaacaggactctaaagactctacatactccctgtcctccacactgaccctctccaaggccgactatgagaaacacaaggtttacgcatgcgaggtcacacaccagggactctcctctcccgtgaccaagagcttcaaccggggagaatgc

SEQ ID NO: 47 - protein, 446 aa, Artificial Sequence
  amino acid sequences of 28H1-Fc9
EVQLLESGGGLVQPGGSLRLSCAASGFTFSSHAMSWVRQAPGKGLEWVSAIWASGEQYYADSVKGRFTISRDNSKNTLYLQMNSLRAQDTAVYYCAKGWLGNFDYWGQGTLVTVSSASTKGPSVFPLAPSSKSTSGGTAALGCLVKDYFPEPVTVSWNSGALTSGVHTFPAVLQSSGLYSLSSVVTVPSSSLGTQTYICNVNHKPSNTKVDKRVEPKSCDKTHTCPPCPAPELLGGPSVFLFPPKPKDTLMISRTPEVTCVVVDVSHEDPEVKFNWYVDGVEVHNAKTKPREEQYNSTYRVVSVLTVLHQDWLNGKEYKCKVSNKALPAPIEKTISKAKGQPREPQVYTLPPSRDELTKNQVSLWCLVKGFYPSDIAVEWESNGQPENNYKTTPPVLDSDGSFFLYSALTVDKSRWQQGNVFSCSVMHEALHNHYTQKSLSLSPGK

SEQ ID NO: 48 - DNA, 1338 bp, Artificial Sequence
  gene of 28H1-Fc9
gaggtgcagctgctggaatcaggaggaggactggtgcagccaggaggatctctgagactgtcttgcgccgccagcggctttacattcagctctcacgccatgtcttgggtccgacaggctccaggcaaaggactggaatgggtgtccgctatttgggccagcggagagcagtactacgccgacagcgtgaagggacggttcaccatcagccgggacaacagcaagaacaccctgtacctgcagatgaacagcctgagggcccaggataccgccgtgtactattgcgccaagggttggctgggcaacttcgactattggggccagggaaccctggtgacagtgtccagcgccagcactaaggggccctctgtgtttccactcgccccttctagcaaaagcacttccggaggaactgccgctctgggctgtctggtgaaagattacttccccgaaccagtcactgtgtcatggaactctggagcactgacatctggagttcacacctttcctgctgtgctgcagagttctggactgtactccctgtcatctgtggtcaccgtgccatcttcatctctggggacccagacctacatctgtaacgtgaaccacaaaccctccaacacaaaagtggacaaacgagtcgaaccaaaatcttgtgacaaaacccacacatgcccaccgtgcccagctccggaactcctgggcggaccgtcagtcttcctcttccccccaaaacccaaggacaccctcatgatctcccggacccctgaggtcacatgcgtggtggtggacgtgagccacgaagaccctgaggtcaagttcaactggtacgtggacggcgtggaggtgcataatgccaagacaaagccgcgggaggagcagtacaacagcacgtaccgtgtggtcagcgtcctcaccgtcctgcaccaggactggctgaatggcaaggagtacaagtgcaaggtctccaacaaagccctcccagcccccatcgagaaaaccatctccaaagccaaagggcagccccgagaaccacaggtgtacaccctgcccccaagtcgggatgagctgaccaagaaccaggtcagcctgtggtgcctggtcaaaggcttctatcccagcgacatcgccgtggagtgggagagcaatgggcagccggagaacaactacaagaccacgcctcccgtgttggactccgacggctccttcttcctctacagcgcgctcaccgtggacaagagcaggtggcagcaggggaacgtcttctcatgctccgtgatgcatgaggctctgcacaaccactacacgcagaagagcctctccctgtctccgggtaaa

SEQ ID NO: 49 - protein, 15 aa, Artificial Sequence
  linker 1
GGGGSGGGGSGGGGS

SEQ ID NO: 50 - protein, 582 aa, Artificial Sequence
  amino acid sequence of (IL10)2-Fc6
SPGQGTQSENSCTHFPGNLPNMLRDLRDAFSRVKTFFQMKDQLDNLLLKESLLEDFKGYLGCQALSEMIQFYLEEVMPQAENQDPDIKAHVNSLGENLKTLRLRLRRCHRFLPCENKSKAVEQVKNAFNKLQEKGIYKAMSEFDIFINYIEAYMTMKIRNGGGGSGGGGSGGGGSSPGQGTQSENSCTHFPGNLPNMLRDLRDAFSRVKTFFQMKDQLDNLLLKESLLEDFKGYLGCQALSEMIQFYLEEVMPQAENQDPDIKAHVNSLGENLKTLRLRLRRCHRFLPCENKSKAVEQVKNAFNKLQEKGIYKAMSEFDIFINYIEAYMTMKIRNGGGGSGGGGSGGGGSEPKSSDKTHTCPPCPAPELLGGPSVFLFPPKPKDTLMISRTPEVTCVVVDVSHEDPEVKFNWYVDGVEVHNAKTKPREEQYNSTYRVVSVLTVLHQDWLNGKEYKCKVSNKALPAPIEKTISKAKGQPREPQVYTLPPSRDELTKNQVSLSCGVKGFYPSDIAVEWESNGQPENNYKTTPPVLDSDGSFKLASKLTVDKSRWQQGNVFSCSVMHEALHNHYTQKSLSLSPGK

SEQ ID NO: 51 - DNA, 1746 bp, Artificial Sequence
  gene of (IL10)2-Fc6
agccccggccagggcacacagtccgagaacagctgcacccactttcccggcaacctgcctaacatgctgagggacctgagggacgccttcagcagggtgaagaccttcttccagatgaaggaccagctggataacctgctgctgaaggagagcctgctggaggacttcaagggctacctgggctgccaggccctgagcgagatgatccagttctacctggaggaggtgatgccccaggccgagaaccaggaccccgacatcaaggcccacgtgaacagcctgggcgagaacctgaagaccctgaggctgaggctgaggaggtgccacaggttcctgccctgtgagaacaaatccaaggccgtggagcaggtgaagaacgccttcaacaagctgcaggaaaagggcatctacaaggccatgagcgagttcgacatctttatcaactatatcgaggcctacatgacaatgaagatcaggaacggcggcggcggcagcgggggcggcggcagcggaggaggcggcagcagccccggccagggcacacagtccgagaacagctgcacccactttcccggcaacctgcctaacatgctgagggacctgagggacgccttcagcagggtgaagaccttcttccagatgaaggaccagctggataacctgctgctgaaggagagcctgctggaggacttcaagggctacctgggctgccaggccctgagcgagatgatccagttctacctggaggaggtgatgccccaggccgagaaccaggaccccgacatcaaggcccacgtgaacagcctgggcgagaacctgaagaccctgaggctgaggctgaggaggtgccacaggttcctgccctgtgagaacaaatccaaggccgtggagcaggtgaagaacgccttcaacaagctgcaggaaaagggcatctacaaggccatgagcgagttcgacatctttatcaactatatcgaggcctacatgacaatgaagatcaggaacggcggcggcggcagcgggggcggcggcagcggaggaggcggcagcgagcctaagtccagcgacaagacccacacctgccccccttgccccgctccggaactcctgggcggaccgtcagtcttcctcttccccccaaaacccaaggacaccctcatgatctcccggacccctgaggtcacatgcgtggtggtggacgtgagccacgaagaccctgaggtcaagttcaactggtacgtggacggcgtggaggtgcataatgccaagacaaagccgcgggaggagcagtacaacagcacgtaccgtgtggtcagcgtcctcaccgtcctgcaccaggactggctgaatggcaaggagtacaagtgcaaggtctccaacaaagccctcccagcccccatcgagaaaaccatctccaaagccaaagggcagccccgagaaccacaggtgtataccctgcccccatcccgggatgagctgaccaagaaccaggtcagcctgagttgcggggtcaaaggcttctatcccagcgacatcgccgtggagtgggagagcaatgggcagccggagaacaactacaagaccacgcctcccgtgttggactccgacggctccttcaagctcgccagcaagctcaccgtggacaagagcaggtggcagcaggggaacgtcttctcatgctccgtgatgcatgaggctctgcacaaccactacacgcagaagagcctctccctgtctccgggtaaa

SEQ ID NO: 52 - protein, 407 aa, Artificial Sequence
  amino acid sequence of IL10-Fc
SPGQGTQSENSCTHFPGNLPNMLRDLRDAFSRVKTFFQMKDQLDNLLLKESLLEDFKGYLGCQALSEMIQFYLEEVMPQAENQDPDIKAHVNSLGENLKTLRLRLRRCHRFLPCENKSKAVEQVKNAFNKLQEKGIYKAMSEFDIFINYIEAYMTMKIRNGGGGSGGGGSGGGGSEPKSSDKTHTCPPCPAPELLGGPSVFLFPPKPKDTLMISRTPEVTCVVVDVSHEDPEVKFNWYVDGVEVHNAKTKPREEQYNSTYRVVSVLTVLHQDWLNGKEYKCKVSNKALPAPIEKTISKAKGQPREPQVYTLPPSRDELTKNQVSLTCLVKGFYPSDIAVEWESNGQPENNYKTTPPVLDSDGSFFLYSKLTVDKSRWQQGNVFSCSVMHEALHNHYTQKSLSLSPGK

SEQ ID NO: 53 - DNA, 1221 bp, Artificial Sequence
  gene of IL10-Fc
agccccggccagggcacacagtccgagaacagctgcacccactttcccggcaacctgcctaacatgctgagggacctgagggacgccttcagcagggtgaagaccttcttccagatgaaggaccagctggataacctgctgctgaaggagagcctgctggaggacttcaagggctacctgggctgccaggccctgagcgagatgatccagttctacctggaggaggtgatgccccaggccgagaaccaggaccccgacatcaaggcccacgtgaacagcctgggcgagaacctgaagaccctgaggctgaggctgaggaggtgccacaggttcctgccctgtgagaacaaatccaaggccgtggagcaggtgaagaacgccttcaacaagctgcaggaaaagggcatctacaaggccatgagcgagttcgacatctttatcaactatatcgaggcctacatgacaatgaagatcaggaacggcggcggcggcagcgggggcggcggcagcggaggaggcggcagcgagcctaagtccagcgacaagacccacacctgccccccttgccccgctccggaactcctgggcggaccgtcagtcttcctcttccccccaaaacccaaggacaccctcatgatctcccggacccctgaggtcacatgcgtggtggtggacgtgagccacgaagaccctgaggtcaagttcaactggtacgtggacggcgtggaggtgcataatgccaagacaaagccgcgggaggagcagtacaacagcacgtaccgtgtggtcagcgtcctcaccgtcctgcaccaggactggctgaatggcaaggagtacaagtgcaaggtctccaacaaagccctcccagcccccatcgagaaaaccatctccaaagccaaagggcagccccgagaaccacaggtgtacaccctgcccccatcccgggatgagctgaccaagaaccaggtcagcctgacctgcctggtcaaaggcttctatcccagcgacatcgccgtggagtgggagagcaatgggcagccggagaacaactacaagaccacgcctcccgtgttggactccgacggctccttcttcctctacagcaagctcaccgtggacaagagcaggtggcagcaggggaacgtcttctcatgctccgtgatgcatgaggctctgcacaaccactacacgcagaagagcctctccctgtctccgggtaaa

SEQ ID NO: 54 - DNA, 681 bp, Artificial Sequence
  gene of Fc9
gacaaaactcacacatgcccaccgtgcccagctccggaactcctgggcggaccgtcagtcttcctcttccccccaaaacccaaggacaccctcatgatctcccggacccctgaggtcacatgcgtggtggtggacgtgagccacgaagaccctgaggtcaagttcaactggtacgtggacggcgtggaggtgcataatgccaagacaaagccgcgggaggagcagtacaacagcacgtaccgtgtggtcagcgtcctcaccgtcctgcaccaggactggctgaatggcaaggagtacaagtgcaaggtctccaacaaagccctcccagcccccatcgagaaaaccatctccaaagccaaagggcagccccgagaaccacaggtgtacaccctgcccccaagtcgggatgagctgaccaagaaccaggtcagcctgtggtgcctggtcaaaggcttctatcccagcgacatcgccgtggagtgggagagcaatgggcagccggagaacaactacaagaccacgcctcccgtgttggactccgacggctccttcttcctctacagcgcgctcaccgtggacaagagcaggtggcagcaggggaacgtcttctcatgctccgtgatgcatgaggctctgcacaaccactacacgcagaagagcctctccctgtctccgggtaaa

SEQ ID NO: 55 - protein, 8 aa, Artificial Sequence
  Kb-binding peptide antigen
SIYRYYGL

SEQ ID NO: 56 - protein, 11 aa, Artificial Sequence
  Cetuximab light chain CDR1
RASQSIGTNIH

SEQ ID NO: 57 - protein, 7 aa, Artificial Sequence
  Cetuximab light chain CDR2
YASESIS

SEQ ID NO: 58 - protein, 9 aa, Artificial Sequence
  Cetuximab light chain CDR3
QQNNNWPTT

SEQ ID NO: 59 - protein, 107 aa, Artificial Sequence
  Cetuximab light chain variable region
DILLTQSPVILSVSPGERVSFSCRASQSIGTNIHWYQQRTNGSPRLLIKYASESISGIPSRFSGSGSGTDFTLSINSVESEDIADYYCQQNNNWPTTFGAGTKLELK

SEQ ID NO: 60 - protein, 5 aa, Artificial Sequence
  Cetuximab heavy chain CDR1
NYGVH

SEQ ID NO: 61 - protein, 16 aa, Artificial Sequence
  Cetuximab heavy chain CDR2
VIWSGGNTDYNTPFTS

SEQ ID NO: 62 - protein, 11 aa, Artificial Sequence
  Cetuximab heavy chain CDR3
ALTYYDYEFAY

SEQ ID NO: 63 - protein, 119 aa, Artificial Sequence
  Cetuximab heavy chain variable region
QVQLKQSGPGLVQPSQSLSITCTVSGFSLTNYGVHWVRQSPGKGLEWLGVIWSGGNTDYNTPFTSRLSINKDNSKSQVFFKMNSLQSNDTAIYYCARALTYYDYEFAYWGQGTLVTVSA

SEQ ID NO: 64 - protein, 11 aa, Artificial Sequence
  Trastuzumab light chain CDR1
RASQDVNTAVA

SEQ ID NO: 65 - protein, 7 aa, Artificial Sequence
  Trastuzumab light chain CDR2
SASFLYS

SEQ ID NO: 66 - protein, 9 aa, Artificial Sequence
  Trastuzumab light chain CDR3
QQHYTTPPT

SEQ ID NO: 67 - protein, 107 aa, Artificial Sequence [sequence omitted]

SEQ ID NO: 68 - protein, 5 aa, Artificial Sequence
  Trastuzumab heavy chain CDR1
DTYIH

SEQ ID NO: 69 - protein, 17 aa, Artificial Sequence
  Trastuzumab heavy chain CDR2
RIYPTNGYTRYADSVKG

SEQ ID NO: 70 - protein, 11 aa, Artificial Sequence
  Trastuzumab heavy chain CDR3
WGGDGFYAMDY

SEQ ID NO: 71 - protein, 120 aa, Artificial Sequence [sequence omitted]

SEQ ID NO: 72 - protein, 6 aa, Artificial Sequence
  28H1 light chain CDR1
SRSYLA

SEQ ID NO: 73 - protein, 7 aa, Artificial Sequence
  28H1 light chain CDR2
GASTRAT

SEQ ID NO: 74 - protein, 9 aa, Artificial Sequence
  28H1 light chain CDR3
QQGQVIPPT

SEQ ID NO: 75 - protein, 108 aa, Artificial Sequence
  28H1 light chain variable region
EIVLTQSPGTLSLSPGERATLSCRASQSVSRSYLAWYQQKPGQAPRLLIIGASTRATGIPDRFSGSGSGTDFTLTISRLEPEDFAVYYCQQGQVIPPTFGQGTKVEIK

SEQ ID NO: 76 - protein, 5 aa, Artificial Sequence
  28H1 heavy chain CDR1
SHAMS

SEQ ID NO: 77 - protein, 16 aa, Artificial Sequence
  28H1 heavy chain CDR2
AIWASGEQYYADSVKG

SEQ ID NO: 78 - protein, 8 aa, Artificial Sequence
  28H1 heavy chain CDR3
GWLGNFDY

SEQ ID NO: 79 - protein, 116 aa, Artificial Sequence
  28H1 heavy chain variable region
EVQLLESGGGLVQPGGSLRLSCAASGFTFSSHAMSWVRQAPGKGLEWVSAIWASGEQYYADSVKGRFTISRDNSKNTLYLQMNSLRAQDTAVYYCAKGWLGNFDYWGQGTLVTVSS

SEQ ID NO: 80 - protein, 160 aa, Artificial Sequence
  IL10
SPGQGTQSENSCTHFPGNLPNMLRDLRDAFSRVKTFFQMKDQLDNLLLKESLLEDFKGYLGCQALSEMIQFYLEEVMPQAENQDPDIKAHVNSLGENLKTLRLRLRRCHRFLPCENKSKAVEQVKNAFNKLQEKGIYKAMSEFDIFINYIEAYMTMKIRN

SEQ ID NO: 81 - DNA, 480 bp, Artificial Sequence
  gene of IL10
agccccggccagggcacacagtccgagaacagctgcacccactttcccggcaacctgcctaacatgctgagggacctgagggacgccttcagcagggtgaagaccttcttccagatgaaggaccagctggataacctgctgctgaaggagagcctgctggaggacttcaagggctacctgggctgccaggccctgagcgagatgatccagttctacctggaggaggtgatgccccaggccgagaaccaggaccccgacatcaaggcccacgtgaacagcctgggcgagaacctgaagaccctgaggctgaggctgaggaggtgccacaggttcctgccctgtgagaacaaatccaaggccgtggagcaggtgaagaacgccttcaacaagctgcaggaaaagggcatctacaaggccatgagcgagttcgacatctttatcaactatatcgaggcctacatgacaatgaagatcaggaac

SEQ ID NO: 82 - protein, 335 aa, Artificial Sequence
  (IL10)2
SPGQGTQSENSCTHFPGNLPNMLRDLRDAFSRVKTFFQMKDQLDNLLLKESLLEDFKGYLGCQALSEMIQFYLEEVMPQAENQDPDIKAHVNSLGENLKTLRLRLRRCHRFLPCENKSKAVEQVKNAFNKLQEKGIYKAMSEFDIFINYIEAYMTMKIRNGGGGSGGGGSGGGGSSPGQGTQSENSCTHFPGNLPNMLRDLRDAFSRVKTFFQMKDQLDNLLLKESLLEDFKGYLGCQALSEMIQFYLEEVMPQAENQDPDIKAHVNSLGENLKTLRLRLRRCHRFLPCENKSKAVEQVKNAFNKLQEKGIYKAMSEFDIFINYIEAYMTMKIRN

SEQ ID NO: 83 - DNA, 1005 bp, Artificial Sequence
  gene of (IL10)2
agccccggccagggcacacagtccgagaacagctgcacccactttcccggcaacctgcctaacatgctgagggacctgagggacgccttcagcagggtgaagaccttcttccagatgaaggaccagctggataacctgctgctgaaggagagcctgctggaggacttcaagggctacctgggctgccaggccctgagcgagatgatccagttctacctggaggaggtgatgccccaggccgagaaccaggaccccgacatcaaggcccacgtgaacagcctgggcgagaacctgaagaccctgaggctgaggctgaggaggtgccacaggttcctgccctgtgagaacaaatccaaggccgtggagcaggtgaagaacgccttcaacaagctgcaggaaaagggcatctacaaggccatgagcgagttcgacatctttatcaactatatcgaggcctacatgacaatgaagatcaggaacggcggcggcggcagcgggggcggcggcagcggaggaggcggcagcagccccggccagggcacacagtccgagaacagctgcacccactttcccggcaacctgcctaacatgctgagggacctgagggacgccttcagcagggtgaagaccttcttccagatgaaggaccagctggataacctgctgctgaaggagagcctgctggaggacttcaagggctacctgggctgccaggccctgagcgagatgatccagttctacctggaggaggtgatgccccaggccgagaaccaggaccccgacatcaaggcccacgtgaacagcctgggcgagaacctgaagaccctgaggctgaggctgaggaggtgccacaggttcctgccctgtgagaacaaatccaaggccgtggagcaggtgaagaacgccttcaacaagctgcaggaaaagggcatctacaaggccatgagcgagttcgacatctttatcaactatatcgaggcctacatgacaatgaagatcaggaac

SEQ ID NO: 84 - protein, 11 aa, Artificial Sequence
  Pertuzumab light chain CDR1
KASQDVSIGVA

SEQ ID NO: 85 - protein, 7 aa, Artificial Sequence
  Pertuzumab light chain CDR2
SASYRYT

SEQ ID NO: 86 - protein, 9 aa, Artificial Sequence
  Pertuzumab light chain CDR3
QQYYIYPYT

SEQ ID NO: 87 - protein, 107 aa, Artificial Sequence [sequence omitted]

SEQ ID NO: 88 - protein, 5 aa, Artificial Sequence
  Pertuzumab heavy chain CDR1
DYTMD

SEQ ID NO: 89 - protein, 17 aa, Artificial Sequence
  Pertuzumab heavy chain CDR2
DVNPNSGGSIYNQRFKG

SEQ ID NO: 90 - protein, 10 aa, Artificial Sequence
  Pertuzumab heavy chain CDR3
NLGPSFYFDY

SEQ ID NO: 91 - protein, 119 aa, Artificial Sequence [sequence omitted]